European Patent Specification EP 3 806 898 B1, published October 8, 2025. Title: GREMLIN-1 ANTAGONIST FOR THE PREVENTION AND TREATMENT OF CANCER. Applicant: UCB Biopharma SPRL Oxford University Innovation Limited The University of Adelaide. The sequence listing filed with the application follows.

SEQUENCE LISTING (43 sequences)

SEQ ID NO: 1 - protein, 184 aa, Homo sapiens
MSRTAYTVGALLLLLGTLLPAAEGKKKGSQGAIPPPDKAQHNDSEQTQSPQQPGSRNRGRGQGRGTAMPGEEVLESSQEALHVTERKYLKRDWCKTQPLKQTIHEEGCNSRTIINRFCYGQCNSFYIPRHIRKEEGSFQSCSFCKPKKFTTMMVTLNCPELQPPTKKKRVTRVKQCRCISIDLD

SEQ ID NO: 2 - protein, 139 aa, Artificial Sequence
  Human truncated Gremlin-1 used in crystallography with N-terminal tag
MGSSHHHHHHSSGENLYFQGSAMPGEEVLESSQEALHVTERKYLKRDWCKTQPLKQTIHEEGCNSRTIINRFCYGQCNSFYIPRHIRKEEGSFQSCSFCKPKKFTTMMVTLNCPELQPPTKKKRVTRVKQCRCISIDLD

SEQ ID NO: 3 - protein, 10 aa, Artificial Sequence
  Ab7326 HCDR1 combined Kabat & Chothia
GYTFTDYYMH

SEQ ID NO: 4 - protein, 5 aa, Artificial Sequence
  Ab7326 HCDR1 Kabat
DYYMH

SEQ ID NO: 5 - protein, 17 aa, Artificial Sequence
  Ab7326 HCDR2 Kabat
LVDPEDGETIYAEKFQG

SEQ ID NO: 6 - protein, 15 aa, Artificial Sequence
  Ab7326 HCDR3 Kabat
DARGSGSYYPNHFDY

SEQ ID NO: 7 - protein, 17 aa, Artificial Sequence
  Ab7326 LCDR1 Kabat
KSSQSVLYSSNNKNYLA

SEQ ID NO: 8 - protein, 7 aa, Artificial Sequence
  Ab7326 LCDR2 Kabat
WASTRES

SEQ ID NO: 9 - protein, 8 aa, Artificial Sequence
  Ab7326 LCDR3 Kabat
QQYYDTPT

SEQ ID NO: 10 - protein, 124 aa, Artificial Sequence
  Ab7326 Heavy chain variable region variant 1
QVQLVESGAEVKKPGATVKISCKVSGYTFTDYYMHWVQQAPGKGLEWMGLVDPEDGETIYAEKFQGRVTITADTSTDTAYMELSSLRSEDTAVYYCATDARGSGSYYPNHFDYWGQGTLVTVSS

SEQ ID NO: 11 - protein, 112 aa, Artificial Sequence
  Ab7326 Light chain variable region variant 1
DIVMTQSPDSLAVSLGERATINCKSSQSVLYSSNNKNYLAWYQQKPGQPPKLLIYWASTRESGVPDRFSGSGSGTDFTLTINSLQAEDVAVYFCQQYYDTPTFGQGTRLEIK

SEQ ID NO: 12 - protein, 124 aa, Artificial Sequence
  Ab7326 Heavy chain variable region variant 2
QVQLVQSGAEVKKPGATVKISCKVSGYTFTDYYMHWVQQAPGKGLEWMGLVDPEDGETIYAEKFQGRVTITADTSTDTAYMELSSLRSEDTAVYYCATDARGSGSYYPNHFDYWGQGTLVTVSS

SEQ ID NO: 13 - protein, 112 aa, Artificial Sequence
  Ab7326 Light chain variable region variant 2
DIVMTQTPDSLAVSLGERATINCKSSQSVLYSSNNKNYLAWYQQKPGQPPKLLIYWASTRESGVPDRFSGSGSGTDFTLTINSLQAEDVAVYFCQQYYDTPTFGQGTRLEIK

SEQ ID NO: 14 - protein, 448 aa, Artificial Sequence
  Mouse full length IgG1 heavy chain variant 1
QVQLVESGAEVKKPGATVKISCKVSGYTFTDYYMHWVQQAPGKGLEWMGLVDPEDGETIYAEKFQGRVTITADTSTDTAYMELSSLRSEDTAVYYCATDARGSGSYYPNHFDYWGQGTLVTVSSAKTTPPSVYPLAPGSAAQTNSMVTLGCLVKGYFPEPVTVTWNSGSLSSGVHTFPAVLQSDLYTLSSSVTVPSSTWPSETVTCNVAHPASSTKVDKKIVPRDCGCKPCICTVPEVSSVFIFPPKPKDVLTITLTPKVTCVVVDISKDDPEVQFSWFVDDVEVHTAQTQPREEQFNSTFRSVSELPIMHQDWLNGKEFKCRVNSAAFPAPIEKTISKTKGRPKAPQVYTIPPPKEQMAKDKVSLTCMITDFFPEDITVEWQWNGQPAENYKNTQPIMDTDGSYFVYSKLNVQKSNWEAGNTFTCSVLHEGLHNHHTEKSLSHSPGK

SEQ ID NO: 15 - protein, 219 aa, Artificial Sequence
  Mouse full length IgG1 light chain variant 1
DIVMTQSPDSLAVSLGERATINCKSSQSVLYSSNNKNYLAWYQQKPGQPPKLLIYWASTRESGVPDRFSGSGSGTDFTLTINSLQAEDVAVYFCQQYYDTPTFGQGTRLEIKRTDAAPTVSIFPPSSEQLTSGGASVVCFLNNFYPKDINVKWKIDGSERQNGVLNSWTDQDSKDSTYSMSSTLTLTKDEYERHNSYTCEATHKTSTSPIVKSFNRNEC

SEQ ID NO: 16 - protein, 454 aa, Artificial Sequence
  Human full length IgG1 heavy chain variant 2
QVQLVQSGAEVKKPGATVKISCKVSGYTFTDYYMHWVQQAPGKGLEWMGLVDPEDGETIYAEKFQGRVTITADTSTDTAYMELSSLRSEDTAVYYCATDARGSGSYYPNHFDYWGQGTLVTVSSASTKGPSVFPLAPSSKSTSGGTAALGCLVKDYFPEPVTVSWNSGALTSGVHTFPAVLQSSGLYSLSSVVTVPSSSLGTQTYICNVNHKPSNTKVDKKVEPKSCDKTHTCPPCPAPELLGGPSVFLFPPKPKDTLMISRTPEVTCVVVDVSHEDPEVKFNWYVDGVEVHNAKTKPREEQYNSTYRVVSVLTVLHQDWLNGKEYKCKVSNKALPAPIEKTISKAKGQPREPQVYTLPPSRDELTKNQVSLTCLVKGFYPSDIAVEWESNGQPENNYKTTPPVLDSDGSFFLYSKLTVDKSRWQQGNVFSCSVMHEALHNHYTQKSLSLSPGK

SEQ ID NO: 17 - protein, 219 aa, Artificial Sequence
  Human full length IgG1 light chain variant 2
DIVMTQTPDSLAVSLGERATINCKSSQSVLYSSNNKNYLAWYQQKPGQPPKLLIYWASTRESGVPDRFSGSGSGTDFTLTINSLQAEDVAVYFCQQYYDTPTFGQGTRLEIKRTVAAPSVFIFPPSDEQLKSGTASVVCLLNNFYPREAKVQWKVDNALQSGNSQESVTEQDSKDSTYSLSSTLTLSKADYEKHKVYACEVTHQGLSSPVTKSFNRGEC

SEQ ID NO: 18 - protein, 227 aa, Artificial Sequence
  Fab heavy chain variant 1
QVQLVESGAEVKKPGATVKISCKVSGYTFTDYYMHWVQQAPGKGLEWMGLVDPEDGETIYAEKFQGRVTITADTSTDTAYMELSSLRSEDTAVYYCATDARGSGSYYPNHFDYWGQGTLVTVSSASTKGPSVFPLAPSSKSTSGGTAALGCLVKDYFPEPVTVSWNSGALTSGVHTFPAVLQSSGLYSLSSVVTVPSSSLGTQTYICNVNHKPSNTKVDKKVEPKSC

SEQ ID NO: 19 - protein, 219 aa, Artificial Sequence
  Fab light chain variant 1
DIVMTQSPDSLAVSLGERATINCKSSQSVLYSSNNKNYLAWYQQKPGQPPKLLIYWASTRESGVPDRFSGSGSGTDFTLTINSLQAEDVAVYFCQQYYDTPTFGQGTRLEIKRTVAAPSVFIFPPSDEQLKSGTASVVCLLNNFYPREAKVQWKVDNALQSGNSQESVTEQDSKDSTYSLSSTLTLSKADYEKHKVYACEVTHQGLSSPVTKSFNRGEC

SEQ ID NO: 20 - protein, 118 aa, Artificial Sequence
  Human truncated Gremlin-1 used in crystallography without N-terminal tag
AMPGEEVLESSQEALHVTERKYLKRDWCKTQPLKQTIHEEGCNSRTIINRFCYGQCNSFYIPRHIRKEEGSFQSCSFCKPKKFTTMMVTLNCPELQPPTKKKRVTRVKQCRCISIDLD

SEQ ID NO: 21 - protein, 160 aa, Artificial Sequence
  Mature Gremlin-1 sequence of SEQ ID NO: 1 lacking the signal peptide of amino acids 1-21
KKKGSQGAIPPPDKAQHNDSEQTQSPQQPGSRNRGRGQGRGTAMPGEEVLESSQEALHVTERKYLKRDWCKTQPLKQTIHEEGCNSRTIINRFCYGQCNSFYIPRHIRKEEGSFQSCSFCKPKKFTTMMVTLNCPELQPPTKKKRVTRVKQCRCISIDLD

SEQ ID NO: 22 - protein, 451 aa, Artificial Sequence
  Human IgG4P heavy chain variant 1
QVQLVESGAEVKKPGATVKISCKVSGYTFTDYYMHWVQQAPGKGLEWMGLVDPEDGETIYAEKFQGRVTITADTSTDTAYMELSSLRSEDTAVYYCATDARGSGSYYPNHFDYWGQGTLVTVSSASTKGPSVFPLAPCSRSTSESTAALGCLVKDYFPEPVTVSWNSGALTSGVHTFPAVLQSSGLYSLSSVVTVPSSSLGTKTYTCNVDHKPSNTKVDKRVESKYGPPCPPCPAPEFLGGPSVFLFPPKPKDTLMISRTPEVTCVVVDVSQEDPEVQFNWYVDGVEVHNAKTKPREEQFNSTYRVVSVLTVLHQDWLNGKEYKCKVSNKGLPSSIEKTISKAKGQPREPQVYTLPPSQEEMTKNQVSLTCLVKGFYPSDIAVEWESNGQPENNYKTTPPVLDSDGSFFLYSRLTVDKSRWQEGNVFSCSVMHEALHNHYTQKSLSLSLGK

SEQ ID NO: 23 - protein, 219 aa, Artificial Sequence; identical to SEQ ID NO: 19
  Human IgG4P light chain variant 1

SEQ ID NO: 24 - DNA, 1362 bp, Artificial Sequence
  Human IgG1 heavy chain DNA variant 1
caagtgcaactggtggaatccggggccgaagtgaaaaagcccggagccactgtgaagatctcttgcaaagtgtccggctacaccttcaccgactattacatgcactgggtccagcaggcacctgggaagggccttgagtggatgggtctggtcgatcccgaggacggcgaaactatctacgccgagaagttccagggtcgcgtcaccatcaccgccgacacttccaccgacaccgcgtacatggagctgtccagcttgaggtccgaggacacagccgtgtactactgcgccacggatgctcggggaagcggcagctactacccgaaccacttcgactactggggacagggcactctcgtgactgtctcgagcgcttctacaaagggcccctccgtgttcccgctcgctccatcatcgaagtctaccagcggaggcactgcggctctcggttgcctcgtgaaggactacttcccggagccggtgaccgtgtcgtggaacagcggagccctgaccagcggggtgcacacctttccggccgtcttgcagtcaagcggcctttactccctgtcatcagtggtgactgtcccgtccagctcattgggaacccaaacctacatctgcaatgtgaatcacaaacctagcaacaccaaggttgacaagaaagtcgagcccaaatcgtgtgacaagactcacacttgtccgccgtgcccggcacccgaactgctgggaggtcccagcgtctttctgttccctccaaagccgaaagacacgctgatgatctcccgcaccccggaggtcacttgcgtggtcgtggacgtgtcacatgaggacccagaggtgaagttcaattggtacgtggatggcgtcgaagtccacaatgccaaaactaagcccagagaagaacagtacaattcgacctaccgcgtcgtgtccgtgctcacggtgttgcatcaggattggctgaacgggaaggaatacaagtgcaaagtgtccaacaaggcgctgccggcaccgatcgagaaaactatctccaaagcgaagggacagcctagggaacctcaagtctacacgctgccaccatcacgggatgaactgactaagaatcaagtctcactgacttgtctggtgaaggggttttaccctagcgacattgccgtggagtgggaatccaacggccagccagagaacaactacaagactacccctccagtgctcgactcggatggatcgttcttcctttactcgaagctcaccgtggataagtcccggtggcagcagggaaacgtgttctcctgctcggtgatgcatgaagccctccataaccactatacccaaaagtcgctgtccctgtcgccgggaaag

SEQ ID NO: 25 - DNA, 657 bp, Artificial Sequence
  Human IgG1 light chain DNA variant 1
gacattgtgatgacccagtcccccgattcgcttgcggtgtccctgggagaacgggccaccattaactgcaagagctcacagtccgtcctgtattcatcgaacaacaagaattacctcgcatggtatcagcagaagcctggacagcctcccaagctgctcatctactgggctagcacccgcgaatccggggtgccggatagattctccggatcgggttcgggcactgacttcactctgactatcaactcactgcaagccgaggatgtcgcggtgtacttctgtcagcagtactacgacaccccgacctttggacaaggcaccagactggagattaagcgtacggtggccgctccctccgtgttcatcttcccaccctccgacgagcagctgaagtccggcaccgcctccgtcgtgtgcctgctgaacaacttctacccccgcgaggccaaggtgcagtggaaggtggacaacgccctgcagtccggcaactcccaggaatccgtcaccgagcaggactccaaggacagcacctactccctgtcctccaccctgaccctgtccaaggccgactacgagaagcacaaggtgtacgcctgcgaagtgacccaccagggcctgtccagccccgtgaccaagtccttcaaccggggcgagtgc

SEQ ID NO: 26 - DNA, 1353 bp, Artificial Sequence
  Human IgG4P heavy chain DNA variant 1
caagtgcaactggtggaatccggggccgaagtgaaaaagcccggagccactgtgaagatctcttgcaaagtgtccggctacaccttcaccgactattacatgcactgggtccagcaggcacctgggaagggccttgagtggatgggtctggtcgatcccgaggacggcgaaactatctacgccgagaagttccagggtcgcgtcaccatcaccgccgacacttccaccgacaccgcgtacatggagctgtccagcttgaggtccgaggacacagccgtgtactactgcgccacggatgctcggggaagcggcagctactacccgaaccacttcgactactggggacagggcactctcgtgactgtctcgagcgcttctacaaagggcccctccgtgttccctctggccccttgctcccggtccacctccgagtctaccgccgctctgggctgcctggtcaaggactacttccccgagcccgtgacagtgtcctggaactctggcgccctgacctccggcgtgcacaccttccctgccgtgctgcagtcctccggcctgtactccctgtcctccgtcgtgaccgtgccctcctccagcctgggcaccaagacctacacctgtaacgtggaccacaagccctccaacaccaaggtggacaagcgggtggaatctaagtacggccctccctgccccccctgccctgcccctgaatttctgggcggaccttccgtgttcctgttccccccaaagcccaaggacaccctgatgatctcccggacccccgaagtgacctgcgtggtggtggacgtgtcccaggaagatcccgaggtccagttcaattggtacgtggacggcgtggaagtgcacaatgccaagaccaagcccagagaggaacagttcaactccacctaccgggtggtgtccgtgctgaccgtgctgcaccaggactggctgaacggcaaagagtacaagtgcaaggtgtccaacaagggcctgccctccagcatcgaaaagaccatctccaaggccaagggccagccccgcgagccccaggtgtacaccctgccccctagccaggaagagatgaccaagaaccaggtgtccctgacctgtctggtcaagggcttctacccctccgacattgccgtggaatgggagtccaacggccagcccgagaacaactacaagaccaccccccctgtgctggacagcgacggctccttcttcctgtactctcggctgaccgtggacaagtcccggtggcaggaaggcaacgtcttctcctgctccgtgatgcacgaggccctgcacaaccactacacccagaagtccctgtccctgagcctgggcaag

SEQ ID NO: 27 - DNA, 657 bp, Artificial Sequence; identical to SEQ ID NO: 25
  Human IgG4P light chain DNA variant 1

SEQ ID NO: 28 - protein, 448 aa, Artificial Sequence
  Mouse full length IgG1 heavy chain variant 2
QVQLVQSGAEVKKPGATVKISCKVSGYTFTDYYMHWVQQAPGKGLEWMGLVDPEDGETIYAEKFQGRVTITADTSTDTAYMELSSLRSEDTAVYYCATDARGSGSYYPNHFDYWGQGTLVTVSSAKTTPPSVYPLAPGSAAQTNSMVTLGCLVKGYFPEPVTVTWNSGSLSSGVHTFPAVLQSDLYTLSSSVTVPSSTWPSETVTCNVAHPASSTKVDKKIVPRDCGCKPCICTVPEVSSVFIFPPKPKDVLTITLTPKVTCVVVDISKDDPEVQFSWFVDDVEVHTAQTQPREEQFNSTFRSVSELPIMHQDWLNGKEFKCRVNSAAFPAPIEKTISKTKGRPKAPQVYTIPPPKEQMAKDKVSLTCMITDFFPEDITVEWQWNGQPAENYKNTQPIMDTDGSYFVYSKLNVQKSNWEAGNTFTCSVLHEGLHNHHTEKSLSHSPGK

SEQ ID NO: 29 - protein, 219 aa, Artificial Sequence
  Mouse full length IgG1 light chain variant 2
DIVMTQTPDSLAVSLGERATINCKSSQSVLYSSNNKNYLAWYQQKPGQPPKLLIYWASTRESGVPDRFSGSGSGTDFTLTINSLQAEDVAVYFCQQYYDTPTFGQGTRLEIKRTDAAPTVSIFPPSSEQLTSGGASVVCFLNNFYPKDINVKWKIDGSERQNGVLNSWTDQDSKDSTYSMSSTLTLTKDEYERHNSYTCEATHKTSTSPIVKSFNRNEC

SEQ ID NO: 30 - protein, 454 aa, Artificial Sequence
  Human full length IgG1 heavy chain variant 1
QVQLVESGAEVKKPGATVKISCKVSGYTFTDYYMHWVQQAPGKGLEWMGLVDPEDGETIYAEKFQGRVTITADTSTDTAYMELSSLRSEDTAVYYCATDARGSGSYYPNHFDYWGQGTLVTVSSASTKGPSVFPLAPSSKSTSGGTAALGCLVKDYFPEPVTVSWNSGALTSGVHTFPAVLQSSGLYSLSSVVTVPSSSLGTQTYICNVNHKPSNTKVDKKVEPKSCDKTHTCPPCPAPELLGGPSVFLFPPKPKDTLMISRTPEVTCVVVDVSHEDPEVKFNWYVDGVEVHNAKTKPREEQYNSTYRVVSVLTVLHQDWLNGKEYKCKVSNKALPAPIEKTISKAKGQPREPQVYTLPPSRDELTKNQVSLTCLVKGFYPSDIAVEWESNGQPENNYKTTPPVLDSDGSFFLYSKLTVDKSRWQQGNVFSCSVMHEALHNHYTQKSLSLSPGK

SEQ ID NO: 31 - protein, 219 aa, Artificial Sequence; identical to SEQ ID NO: 19
  Human full length IgG1 light chain variant 1

SEQ ID NO: 32 - protein, 227 aa, Artificial Sequence
  Fab heavy chain variant 2
QVQLVQSGAEVKKPGATVKISCKVSGYTFTDYYMHWVQQAPGKGLEWMGLVDPEDGETIYAEKFQGRVTITADTSTDTAYMELSSLRSEDTAVYYCATDARGSGSYYPNHFDYWGQGTLVTVSSASTKGPSVFPLAPSSKSTSGGTAALGCLVKDYFPEPVTVSWNSGALTSGVHTFPAVLQSSGLYSLSSVVTVPSSSLGTQTYICNVNHKPSNTKVDKKVEPKSC

SEQ ID NO: 33 - protein, 219 aa, Artificial Sequence; identical to SEQ ID NO: 17
  Fab light chain variant 2

SEQ ID NO: 34 - protein, 451 aa, Artificial Sequence
  Human IgG4P heavy chain variant 2
QVQLVQSGAEVKKPGATVKISCKVSGYTFTDYYMHWVQQAPGKGLEWMGLVDPEDGETIYAEKFQGRVTITADTSTDTAYMELSSLRSEDTAVYYCATDARGSGSYYPNHFDYWGQGTLVTVSSASTKGPSVFPLAPCSRSTSESTAALGCLVKDYFPEPVTVSWNSGALTSGVHTFPAVLQSSGLYSLSSVVTVPSSSLGTKTYTCNVDHKPSNTKVDKRVESKYGPPCPPCPAPEFLGGPSVFLFPPKPKDTLMISRTPEVTCVVVDVSQEDPEVQFNWYVDGVEVHNAKTKPREEQFNSTYRVVSVLTVLHQDWLNGKEYKCKVSNKGLPSSIEKTISKAKGQPREPQVYTLPPSQEEMTKNQVSLTCLVKGFYPSDIAVEWESNGQPENNYKTTPPVLDSDGSFFLYSRLTVDKSRWQEGNVFSCSVMHEALHNHYTQKSLSLSLGK

SEQ ID NO: 35 - protein, 219 aa, Artificial Sequence; identical to SEQ ID NO: 17
  Human IgG4P light chain variant 2

SEQ ID NO: 36 - DNA, 16654 bp, Homo sapiens
actcggtgcgccttccgcggaccgggcgacccagtgcacggccgccgcgtcactctcggtcccgctgaccccgcgccgagccccggcggctctggccgcggccgcactcagcgccacgcgtcgaaagcgcaggccccgaggacccgccgcactgacaggtgagcgcggacgcacccggcagggatgtgagtgggcggagggaagagggccgcaaaccaacccaggacccgctcagttccacgcgcggcagccctccgtgcgcgcaggctcgggtgcgttgttcgcgggggtgaattgtgaagaaccatcgcggggtccttcctgctgaggccgcggacaccgtgacctcgctgctctgggtctgcagggaaacgtaggaaaaaaagttgtcaggagcgggcaggatgacccccacatcccgtttccacctcccggaggcccccgaacacgctcctggtgctggtggcagcagcgcctggcagacgcgcccgcttagcgagggcgcgaagtccaggccgccagagcgcaggagcatccggacctgctagtcggccgctgactgcgcggcgagttgccttgagagggtcccatgtgcttggggcgccgcgctgggtctgggggcgtcttggggcgcccattggagtccgcgggttggagcatccggagaatccatgatgtgtgcatttgccgatccccgaggtgagatggagactggcaagggcagagccgctgtgttcagccacagcggaaaaccgaacggtgggtaatccgacagctgcggtgcggggcgcggccctggccgcggggtccagcgaacccgcagtgctcacaaggcagacaccacacgcgctcgcggaccggccacgcactcgcgggcgctcgcttctctactccagcctcttccccgccccgcgcacgcccgagctgaatggtagacgttctggcgccgggcagcggccaccggctggttcccacttccgcgcgcaccccttaaactgtgttctagaggccccagcctcgccttgcagcgcctcactagctcctgaggactagggactggcggctgaggcgggttggcggctgcaacgagctgggcgtctttcgttctctctcgctgcctggctggctccgctggcccctccacagcttgcggagcaaggccatagcaggggagtgggaggtatattggggctgtcacctccttgctggccggagttatttgtagactacagactccggaagaacagacgcgccaccgctctcgcttggcattgccttcggatcgcagctcctccttgggggtgccccagcttggcgtttatttgcctgcgccaggctctggcgacggtcaccgggccaggcggggagggacggacggcaggtgaccagcctctgctgtgaagaaattcctgcgcgcccggagctgtccctaatgcattcccgggtcgaatccgtctactgccttcccctcctcgaccgactccgaatctcggctcttatagacagaaatacagcctcagcgttaggggttaaaatccccctcttaaacggtccgagggcagagaggtgaccaccgataggtaattggatctcctgctggaaagagcaaatctgagcggtgtgcgcgtctgtttatgttccccttcgagatggtgccaggacacgaactgattaaaacaatctattgtgttaagtgggtcactagggttttaagctgtcccagggaccccagagtagtggcttccttctggctgtacacacaagttaaataaatagcgtagaagaggttaagataaccccattctagggtgaggagtcctctttcatccctagggcttccccctccccttttctctttttttggaaggagggggagcatgagagtcttgagggggggatgtacttttcaaagcaaggagggaaagatcttaagaaaactatatattctcactgccccccaagccaagtctataacagtaggtgatttgattactatctctggataaatggcactgtcaaattgttaatattaactatttcagggatttttagcagggtagtggcagtatgtgtgcgtgtgtgtgtgtgtgtctgtgtgtgtgtgtttaacctccaggtcattgtaggaattagagtcttttgtaaactttgtaatttcacaggtttcctattttcttaaaagttcatttttagtgaaatgttttggtaacccacgctctgtaggaaatccaggttggctaatgcggtctttatgtgagtagttacacagggaaggataaaaaccttttatgtcctacatctctgaatgagggctgcctaccctgtctttgaaactaagccgaagatgccttcagtctgaatggtcaagtattaaaagtgataaaatgcaaagaaatttcatgccgcagacacctcccccaagaactgcttgttgacagcaaagctgtggaacatgttccacaacagagagtaaaggacagccaggaaatataaaccttttatgtaaaggaaaggcaggtgggggacagtggttaggggaggtgactgcagcctctaaccaaaaggcaaccatcaggcaagtgctaccagcccgtgtcttcgatctgcaaggaattttctttagttttaacatatgctcttagaaattcaaagtacaacaggaattcctgggacaagagaaatctttttattcacatgtgaacatgaagatacaaaatagataattattttatttatagcactcttcaaattgtattgcattagaaaacatatccattgacccactgttaaggacagcactgggtgtcaataggacagtggttaaggacctgtgtttggggctagatagaattgggtttaaactgctggctgggctgggcacagtggctcacaccggtaatcccagcactttgggaggccaaggaggacggatcacctgaggtcgggagttcgacaccagcctgaccaacatggaaaaatcccgtctctactaaaaacacaaaattagccaggcatggtggtgcatgcctgcaatcccagctacttgggaggctgaggcaggagaattgcttgaaaccgggaggcggaggttgtggtgagcccagatagcgccattgcattccagcctgggcaacacgagtgaaaactccgtcaaaaaaacaaaacaaaacaaacaaacaaaaaaatgctggctttcccacttatgagctgtgtgaccttggacaaatttccaacttttctgagtgtagattccctgattggtaaaaggaagatgatattatctacctcatattttgttatgaaaaataaatgataaaattgggtcagaaatcagcataatgcctggcacagtaagggcttcaaaataaaaggtagctcttattattagtaatggtgttaggaaaagtagcaatgttatacagaaccaggatatatcacagggcagttctgaaattaaatcctgaatcctggccgggtgaggtggctcacgcttgtaatcctaagcactttcggagactgaggcaggcggatcacgaggtcaggagtttgagaccagcctggccaacacactgaaatcccgtctctactaaaaatacaaaaattagctgggtgtggtggcaggcgcctataatctcagctacttgggaggctgaggcaggagaatcacttgagcccaggaggcggaggttgcagtgagctgatatcgtgccagtgcactccagcctgggtgacatctcttaaaaaaaaaaatcctgaataccacactacgcagtgactaacacatctttcactacagaacagaacctgtaacttggccgtctctcagcagtgctgctcagtgaacatttaataatttattactttctaactcgtttcttgttgacctcaagaattgtacatagtcattaactttcctaagaaaatctttgacaaacatagagctcctgagatatttcacaaccaggtggtctcctccctgtcctatgcaatgttgggccccagcctgatttagccgacctggtcttcagacttgagaggctgtttagggttcttacaacacaaaggggatgagactttatcctctacctgtgtgccaacaagggattcttcttatctccttggtgcaacttgtctgaaaaagaaagtcaacacaattatcttcttaaaagttaaagatcaaattaaaaataagctatagttttcccaaagatttagacctgagaaaaaggaatagatctttctaaaacctggcctgcacttagagcatttgtagtcacttccactatttcttatgctgagagaataatttgatgtcatgcctattgaatgtctttctaaagcttgattcatcaggaggaactgaccagaagtccatgcacagacatttggctttcactgtaattcctactcaaaactccctttcactgattatgagcaggttgcttagctaaaatgagaaatacagcaagaagagggatggaaagagctggcttaaactttcccaaagacatcatgaacactgggaacaggtcatacatataccatttttatttctcagtcctcagtattagaatattgtgttcctagaggctttgtgaaaattggaatacattgccatgacctgcacaggatagaggtggttaatatggcttaccttgcttgtagatgtttactcttgatccctaagggaaactggaaggaaagcatgctgtagagaggacctgctttgagagtatgtgtcctctgggacaagtggaatgaaagagaggatagaggcaaagagaaaaaaaggtggagatggggtgagacttgctggtggacagttgcaaagaaaactcatgatgagaataacatcacatttcttgaagaagctgaactgcattgatgggaagttgaggcagagtttgaaaagaagatatactgtctgcaaaaaagaatcaacggagatgtcaggtatcttgatgcaccctgagtctatgagatgcagcttaatttaatttaatgatatgagtaggccatttcataagtggtggaaattaccataaagtgtttgcagctaatgacggcgcatgaatgatgtcataggaacctaagtctggatgagctatggattgaatttttactatgggacacccttctacatgttgctgtggaaaagaattgtcctcaagaaatgtacatcttctgcatttcctctacatctctgatatttacaaagtgcacattatttggtgatactacaactgggatttcaagtgcacatcactactatttccttcactgaagaatcaagagcagtctgggggtggggagagcttgagtgattgacaaggatgtggcagagccctggttccactatgaattatagttcttaccctgcttactgtcactcatgtagagcagctagtgtgcctcagagcactgctgttctctgagaagctgaggtctcgattgacattcttgaagttggtgtttacttctctctgaataaacaaaggttggcaactcagacatcttacaataagtactaaagatttttgaagaataggtttttaaaaaatgaaaaaacatttcactttccatagctaataaatcttattttgaggaaaatgtacttttctttaaaaaaaaaaaaagcctgtctgtcactctagaccctttggcttagaaggtaggcacactcacatagaaacagaaagtctgtccaaattaaaactgaaaaccacagttgactaattttgaatttatagctctgctgttggcttctgcgatagtattaatttcaatggcttcaattagaaaatgaaacccatagcattccatatgagaacaggtaaaaagtcagggacatttggagttttccaagaaaaagaaagacaagtcttaggaagctctctaggatggaaggaatttgccacactgagagttagacatccaaaggatagcaattggctcttctgctcatgggcactggtgaaggcattttaaaatgcgaagaatggtacctctgtaaatcaatgaggttcataataatcatgcatttaccaaatttttataagcacctgccttgtgccaggcactgagggtaaggtgatgaataagccctcatcaactgtcagactagatatttactcaataacagatgtgaaaatgccaagaaggaaaagttgagtataaagaaagccttaagttggttcagagaaataaaattgcatttttcggatagatgtttatggaatcggccttatgaggtaaacttgtcctatgcagtgaacatacattcccagttagtctcagattggcctctgtgatgacaaactcagagggtcctggtctaggaggggtgaatttgtctggaggccattttcaggaggtatggaggaagactggggcataggcctggggccatcccatgtactcctcctctgaaatggggagcaactgaattgtgttttattttagatcttcgtccaacttgaataccagaaattcgtgaaaccttctcaaattcacactatattttgagaccaggagaaggctccttgagaaattgccacactgtcttatcctagtctctggaaaaattcagtcctgtattataactgggcgtttctcataagtgctttttttttttctttttctttttataatactttaagttctgggatacatgtgcagaatgtgcaggtttgttacataggtatacacgtgccatggtggtttgctgcacccatcaacccatcatctacattaggtatttctcctaatgctaccccttccctagccccccacccctcgacaggccccagtgtttgatgttcccctccctgtgtccatgtgttctcattgttcaactcccacttatgagtgagagcatgcggtgtttggttttctgttcctgtgttagtttgctgagaatgatggtttttggcttcatccacgtccctgcaaaggacatgaactcatcctttttatggctgcatagtattccatggtgtatatgtgccacatttgctttatccagtctatcattgatgagcacttgggttggctccaagtctttgctattatgactagtactgcgataaacatgtgtatatgtgtctttatattagaatgatttataatcctttaggtctatacccagtaataggattcctgggtcaaatggtatttctggttctagatccttgaggaattgccacactgtcttccacaacggttgaactaatttacactcccaccaacagtgtaaaagcattcctatttctccacatcctctccaacatctgttgtttcctgactctttaatgacggccattctaactggcgtgaaatggtatctcattgtggttttgatttgcatttctctaatgaccaccgatgatgagctttttctcatatgtttgctggccccataaatgtcttcttttgagaaatgtctgttcatatcctttgcccactttttgatggggttgtttgcttttttcttgtaaatttgtttgagttcctggtagattctggatattagccctttgtcagatggatagactgcaaaaattttctcccattctgtaggttgcctgttcactctgatggtagtttcttttgccatgcagaagctgtttagtttaattagatccaatttgtcagttttggcttttgttgccattgcttttggtgttttagtcatgaagtctttgcccatgcctatgtcctgaattgtattgccctggttttcttctaggatttttatggttttaggtcttacatttaagtctttaatccatcttgaattaatttttgtataaggtgtaaggaaagggtccagtttcagttttctgcgtatggctagccagttttcccaacgttatttattaaatagggaatcctttccccattgcttgtttttgtcaggtttgtcaaagatcagacggttgtagatgtgtggtgttatttctgaggcctctgttctgttccattggtctgtatatctgctttgataccagtaccgtgctgttttggttactgtagccttgtagtacagtttgaagtcaggtagcgtgatgctttgttctttttgcttaggattgtcttggctatatgggctcttttttggttctatatgaaatttaaagtagttttttcatagacatctatagaactctccaccccaaatcaacagaatatacattcttctcagtatcgcatcacacttattctaaaatgaccacataattagaagtaaaacactcctcagcaaatgcaaaaaacagaaatcctaacagtctgtcagaccccagtgcaatcaaattagaactcaggattaagaaacttactgaaaaccacacaactgcatggaaactgaacaacctgctcctgaatgactactgggtaaataacaaaattaaggcagaaataaataggttctttgaaagaaatgagaacaaagacacaatataccagaatctctgggacacagctaaagcagtgtttagagggaaattgatagcactaaatgcccacaggagaaagcgggacagatctaaaatcgacaccctaatatcacaattaaaagaactagagaaacaagagcaaacaaattcaaaagctagcagaagacaagaaataactaagatcagagcagaactgaaggagatagagacacaaaaaacccttcaaaaaatcaatgaatccaggagctgtttttttttttttgaaaagattaatgaaatagactgctagccaaactaataaaggagaaaagagagaagaatcaaatagacaatagacacaataaaaagtgataaaggggatatcaccactgatcccacagaaatacaaactaccatcagagaatactataaacacctctacgcaaataaactagaaaattgggaagaaatggatacattcctgaacgcatacaccctcccaagactaaaccaggaagaagttgaatccctgaatagaccaatagcaagttctgaaattgaggcagtaattagtagcctaccaaccaaaaaaagcccaggaccagacagattcacagccgaagtctaccagaggtacaaagaggagctagtaccattccttctgaaactattccaaacaatagaaaaagaaggactcctccctaactcattttatgaggccagcatcatcctgataccaaaacctggcagagacacaacataaaggaaattcaggccaatatccctgatgaacattgatgtgaaaatcctcaataaaatactggcagcacatcaaaaagcttacctgccatgatcaagttggcttcatccctgggatgcaaggctggttcaacatacgcaaatcaataaacgtaatcaatcacatacacagaaccaatgacaaaaaccacatgattatctcaatagatgcagaaaaggccttcgataaaattcaacaccccttcaatgctaagaactctcaataaactaggtattgatgaaacatatctcaaaataataagagttatttatgacaaacccacagccagtatcatactgaatgggcaaaagctggaagcattccctttgaaaaccgccacaaggatgacttctctcaccactcctattcaacatactattggaagttctggccagggcaagcaggcaagacaaataaataaagggtattcaaataggaagagaggaagtcaaattgtctctgtttgcagatgacatgattgtatatttagaaaaccccatcatctcagcccaaaatctccttaagctgataagcaacttcagcaaagtctcaggatacaaaatcaatgtgcaaaaatcacaagcattcctatacaccaataatagacaaacagccaaatcatgagtgaactcccattcacaagtgctacaaagaataaaatacctaggaatccaacttacaagggatgtgaaggacctcttcaaggagaactacagaccactgctcaaggtaataagagaggacacaaacaaatggaaaaacattccatgctcatggataggaagaatcaatattatgaaaatggccatactgcccaaaacaatttatagattcaatgccatccccatcaagctaccactgacttccttcacagaattagaaaaaaactactttaaatttcatatggaactgaaaaaagagccggtatagccaagacgatcctaagcaaaaagaaaaaagctggaagcatcatgctacctgacttcaaactatactacaaggctacagtaacaaaaacagcatggtatagtataagtgcttttttttaaaagacaaagtaaagtaatttttttgttgttggggtaaaacaaaagctctgcataaagagcagggatgttgtaacatacactgaccaaaggtgggaaacctacagttggagcagaagctgaatgtcacattatcagctccgaacttataatggtctaaaagtactaggttaatgttggaaagatggtgccatttaaagatatcttaaattcaatatttaattattttaatttgacattatcctagagttgaatggtgtttacttaccatgtgctgttcattagaaaatctagatcctacactgcctttgcgcaaggtagttgctctaataataccaacctgtccagttttggtgggagaaataatgttactgttaagttgcacttagtggttattatgtgtaatactggtattccaaagagagaaggaaaatgtttgctacacagctgtgttcttaggttcagaaaaccacaggagtgggacaggagaaccttcaggattcaggtccgattgttgtgatggccgcaggagggagactgtgaatttgaaactgcatccattgaaaagaaaatccctccacactttaataattctctccgtgccccatggcagcaagtgcttataggccttgctactcaaagcttaataaaaaggcagacctgctgaatcataatctgcatcttaacaatatccccagatattgtctgcactttctttttttttttctttctttctttcttcttttttttgagacagagtctcgctcagtcacccaggctggagtgcagtggcgcgatctcggctcactgcaagctctgactcccgggttcacgccattctcctgccttagactcccgagtagctggcactacaggcgcccgccactacgcccggctaatttttttgtatttttagtagagatggggtttcaccgtgttagccaggatggtctcgatctcctgacctcgtgatccgccgcccatctgggcctcccaaagtgctgggattacaggcgtgagccactgcgcccggccaattgtctgcactttcaagtctaagaagcactgtcccaggaggaaaatctttttagtctgaggcttctctcttgcactctcctttttaaaaatatgctgctccttctccacctttccctcttcttccgccttttctgtctgcctttactacctcccctgaacattcaacttgtagaagagttcccctttctctgaattgcattcttcacttcattcattcttttctctctctgtctatggtttcctattttttgtcggttttccctcacctcacctccttgttattttttgccattgttcacatatcactgccctttcagacccatatctagcttctgacccatccactaatccattgccactaatttattcagcatgcccatgccatttattaatgtaaatatttgcacatacttgttctatcatgcccatttttctaccttttaaattgtatatacacagacacatgtgaatgacatatttcactatttaaaaggtagaaaaatgtatatcgtggtacaaagtgatacattgagtatctgtgcccagtttcaagatgagaataagtgagaggtgaagcctcatgagtcacgtcacctacacgctactgtctttcattccatctgcagtactgccacacatttggttagttctccaattgctgtcacattgacatcgagttggatctgaacagcgtacctggggagacgaagtattggtatctttgcttaaatggagtgatttactgagagacaaagtgacatctttaagatcagatagcaagttactgcaccaggagcgcgacctttcctgttttgttgttttccctctgtcaaatgccttctggtctccatgaatctctccttccacatatgataaaaatgcaaagtctcataagcattcacagctcaggaagcctcaggctagttggggagaaaagactgggaggtttccggaggaatgaagtcctctgagcagagaggttaattcatcttgctgtaaaacaaaatagaaaataagttcccctcaataagtgaacgtaatacaaagacaaatgtggttggtgccagaggccaggaagaagttcttgtgagaataggtgcagagaagagctaggccctggctgagtttaaaccttgacttagtcactgtgggactctgggtgagttactccatggattgatggctgggtcatggagataatagtacctaattcatacaggtactgtgagaagtaaatggaatatttcacgttaagtgtttaacggtgcgtttaaatgctaggtgctattattattaatttttaaattaactttgccatgttttgtgtcttcccctctctgtgcttcctttctttagtatgagccgcacagcctacacggtgggagccctgcttctcctcttggggaccctgctgccggctgctgaagggaaaaagaaagggtcccaaggtgccatccccccgccagacaaggcccagcacaatgactcagagcagactcagtcgccccagcagcctggctccaggaaccgggggcggggccaagggcggggcactgccatgcccggggaggaggtgctggagtccagccaagaggccctgcatgtgacggagcgcaaatacctgaagcgagactggtgcaaaacccagccgcttaagcagaccatccacgaggaaggctgcaacagtcgcaccatcatcaaccgcttctgttacggccagtgcaactctttctacatccccaggcacatccggaaggaggaaggttcctttcagtcctgctccttctgcaagcccaagaaattcactaccatgatggtcacactcaactgccctgaactacagccacctaccaagaagaagagagtcacacgtgtgaagcagtgtcgttgcatatccatcgatttggattaagccaaatccaggtgcacccagcatgtcctaggaatgcagccccaggaagtcccagacctaaaacaaccagattcttacttggcttaaacctagaggccagaagaacccccagctgcctcctggcaggagcctgcttgtgcgtagttcgtgtgcatgagtgtggatgggtgcctgtgggtgtttttagacaccagagaaaacacagtctctgctagagagcactccctattttgtaaacatatctgctttaatggggatgtaccagaaacccacctcaccccggctcacatctaaaggggcggggccgtggtctggttctgactttgtgtttttgtgccctcctggggaccagaatctcctttcggaatgaatgttcatggaagaggctcctctgagggcaagagacctgttttagtgctgcattcgacatggaaaagtccttttaacctgtgcttgcatcctcctttcctcctcctcctcacaatccatctcttcttaagttgatagtgactatgtcagtctaatctcttgtttgccaaggttcctaaattaattcacttaaccatgatgcaaatgtttttcattttgtgaagaccctccagactctgggagaggctggtgtgggcaaggacaagcaggatagtggagtgagaaagggagggtggagggtgaggccaaatcaggtccagcaaaagtcagtagggacattgcagaagcttgaaaggccaataccagaacacaggctgatgcttctgagaaagtcttttcctagtatttaacagaacccaagtgaacagaggagaaatgagattgccagaaagtgattaactttggccgttgcaatctgctcaaacctaacaccaaactgaaaacataaatactgaccactcctatgttcggacccaagcaagttagctaaaccaaaccaactcctctgctttgtccctcaggtggaaaagagaggtagtttagaactctctgcataggggtgggaattaatcaaaaaccgcagaggctgaaattcctaatacctttcctttatcgtggttatagtcagctcatttccattccactatttcccataatgcttctgagagccactaacttgattgataaagatcctgcctctgctgagtgtacctgacagtagtctaagatgagagagtttagggactactctgttttagcaagagatattttgggggtctttttgttttaactattgtcaggagattgggctaaagagaagacgacgagagtaaggaaataaagggaattgcctctggctagagagtagttaggtgttaatacctggtagagatgtaagggatatgacctccctttctttatgtgctcactgaggatctgaggggaccctgttaggagagcatagcatcatgatgtattagctgttcatctgctactggttggatggacataactattgtaactattcagtatttactggtaggcactgtcctctgattaaacttggcctactggcaatggctacttaggattgatctaagggccaaagtgcagggtgggtgaactttattgtactttggatttggttaacctgttttcttcaagcctgaggttttatatacaaactccctgaatactctttttgccttgtatcttctcagcctcctagccaagtcctatgtaatatggaaaacaaacactgcagacttgagattcagttgccgatcaaggctctggcattcagagaacccttgcaactcgagaagctgtttttatttcgtttttgttttgatccagtgctctcccatctaacaactaaacaggagccatttcaaggcgggagatattttaaacacccaaaatgttgggtctgattttcaaacttttaaactcactactgatgattctcacgctaggcgaatttgtccaaacacatagtgtgtgtgttttgtatacactgtatgaccccaccccaaatctttgtattgtccacattctccaacaataaagcacagagtggatttaattaagcacacaaatgctaaggcagaattttgagggtgggagagaagaaaagggaaagaagctgaaaatgtaaaaccacaccagggaggaaaaatgacattcagaaccagcaaacactgaatttctcttgttgttttaactctgccacaagaatgcaatttcgttaacggagatgacttaagttggcagcagtaatcttcttttaggagcttgtaccacagtcttgcacataagtgcagatttggctcaagtaaagagaatttcctcaacactaacttcactgggataatcagcagcgtaactaccctaaaagcatatcactagccaaagagggaaatatctgttcttcttactgtgcctatattaagactagtacaaatgtggtgtgtcttccaactttcattgaaaatgccatatctataccatattttattcgagtcactgatgatgtaatgatatattttttcattattatagtagaatatttttatggcaagatatttgtggtcttgatcatacctattaaaataatgccaaacaccaaatatgaattttatgatgtacactttgtgcttggcattaaaagaaaaaaacacacatcctggaagtctgtaagttgttttttgttactgtaggtcttcaaagttaagagtgtaagtgaaaaatctggaggagaggataatttccactgtgtggaatgtgaatagttaaatgaaaagttatggttatttaatgtaattattacttcaaatcctttggtcactgtgatttcaagcatgttttctttttctcctttatatgactttctctgagttgggcaaagaagaagctgacacaccgtatgttgttagagtcttttatctggtcaggggaaacaaaatcttgacccagctgaacatgtcttcctgagtcagtgcctgaatctttattttttaaattgaatgttccttaaaggttaacatttctaaagcaatattaagaaagactttaaatgttattttggaagacttacgatgcatgtatacaaacgaatagcagataatgatgactagttcacacataaagtccttttaaggagaaaatctaaaatgaaaagtggataaacagaacatttataagtgatcagttaatgcctaagagtgaaagtagttctattgacattcctcaagatatttaatatcaactgcattatgtattatgtctgcttaaatcatttaaaaacggcaaagaattatatagactatgaggtaccttgctgtgtaggaggatgaaaggggagttgatagtctcataaaactaatttggcttcaagtttcatgaatctgtaactagaatttaattttcaccccaataatgttctatatagcctttgctaaagagcaactaataaattaaacctattctttctgtg

SEQ ID NO: 37 - DNA, 555 bp, Homo sapiens
atgagccgcacagcctacacggtgggagccctgcttctcctcttggggaccctgctgccggctgctgaagggaaaaagaaagggtcccaaggtgccatccccccgccagacaaggcccagcacaatgactcagagcagactcagtcgccccagcagcctggctccaggaaccgggggcggggccaagggcggggcactgccatgcccggggaggaggtgctggagtccagccaagaggccctgcatgtgacggagcgcaaatacctgaagcgagactggtgcaaaacccagccgcttaagcagaccatccacgaggaaggctgcaacagtcgcaccatcatcaaccgcttctgttacggccagtgcaactctttctacatccccaggcacatccggaaggaggaaggttcctttcagtcctgctccttctgcaagcccaagaaattcactaccatgatggtcacactcaactgccctgaactacagccacctaccaagaagaagagagtcacacgtgtgaagcagtgtcgttgcatatccatcgatttggattaa

SEQ ID NO: 38 - DNA, 20 bp, Artificial Sequence
  Mouse Grem1 forward primer
gcgcaagtatctgaagcgag

SEQ ID NO: 39 - DNA, 20 bp, Artificial Sequence
  Mouse Grem1 reverse primer
cggttgatgatagtgcggct

SEQ ID NO: 40 - DNA, 21 bp, Artificial Sequence
  Human Grem1 forward primer
aggcccagcacaatgactcag

SEQ ID NO: 41 - DNA, 21 bp, Artificial Sequence
  Human Grem1 reverse primer
gtctcgcttcaggtatttgcg

SEQ ID NO: 42 - DNA, 20 bp, Artificial Sequence
  Beta-actin forward primer
gatcattgctcctcctgagc

SEQ ID NO: 43 - DNA, 22 bp, Artificial Sequence
  Beta-actin reverse primer
gtcatagtccgcctagaagcat